European Patent Application EP 4 289 945 A1, published December 13, 2023. Title: Novel bacteriophage having a specific bactericidal activity against Clostridium perfringens and antibacterial composition comprising the same. Applicant: CJ CheilJedang Corporation. The sequence listing filed with the application follows.

SEQUENCE LISTING (1 sequence)

SEQ ID NO: 1 - DNA, 51670 bp, bacteriophage CJ_CP_20-25
ctttttcttctagtgtactgtttaccatatcgggttacagtgtactctgtactctcatcatctagcttaagaattttaattgtcttagggtcttcaatttcttttatctcttttacgagagctgagtctttaggatcttctacgatctctaaaaaagaatacccaagtccttctctccaatcaactatctcttcaaagacattcttggttggtttatcaaaagacagggtatcaattaattcttccagctgtttatattcagcttccatttctggagtaggttcatctaccttctcaatatacctaatacctattccgaatccagcaatattatttcggtaggcctttttgcattggggtattattgtagactcccttataatcacttctaatagttgggggtcatattcaggggatatctcatcaacttcaattccaagtacactggtttgttgattagatttatccactggatccaaagacttttggatagggtctccacatatacttctggcggatatctttttcaaagttactttacctcctttcttaccttatatatcaaattataaaatccagatggcctcatatttcagggaggattacatcaactccacatatagtgtcaaatacggccattcacatgatttaaaaataactataatttgatacgtttattataacataattcacaaaaatttgtcaacgttttatttttacattattttccagaagattttccgcatatattccccatataaaattatataattattaatgtatactatattactatattaatttatgaaataaattatatagtatatagtatacttatattacatatatataaaggtggtaactctgatatgccttctatatcacattattactaatatagagcctagtcaatttcaaaactgatatctcacatatcagaataaaaattattggctttaataggcatatcagttacttagatttttcttaatttagatccaacaggaaggcaagctaagaatagagagtctgctaagtctggagaatgtagtcctcttttcttcatttcatccttactctccagctttatttgacctttggagttgaatactttaaactttctggtagtcaattctcccacaagatctgtattatctggtagtcttaactcatcatcctccagtaattccttaactacagaggctatatatgtggttgtatcataataaaaggcataagcctgggaccccctctttaatggcataccaaatttacatggtactaccttcaaccagtccagtttttcttcaaattttatctcctttaatctatcagttactcccccacctacaccagtgtcgtctattttcacaactactgctagtttagggaactcaccatgtagggatttagcctttcttagcacttctcctactgttttcatagtgtccttaccttggtaatagataggttcttccacatatccatcaattttggtcataatagaggtcttatctgaaccaaatctagctacgtctacacccatatctatagtaactggttctgtaggtctggttatttcactattaatacctctatatactgtggataattgtataaatatgtcatcttcttctagtgggaagtccccttttaccagacatctgtagacattggactcttctccatactttttccttaacattttatggttttctttatcagttctatcaacttttgtagcgtcaatatgaatacatttaaaattttccttaagactgtggtgagaatcaaagaagatacctgtatttttaacagggttaccaatcaaaattatcttattttcctcatcggatatagtaccaagtaatgcttctagtatctcatcatctattccaggagcctcatcacatataattagcataaactcactatgaagaccaagcatattctcttttctattactagttttacacatagcaaaccaagtcataggactacaattcctagtcatagtagttttatttactgtaaagtaatcttccacaatagttccttgtagccattttgatatttcaggccataatacagatgttaactgtgaaaatgtaggagctgtagcaattaccttacattcaggcctaaaggtcatataccaaattataagacaagcacaggccatggtcttacctaccccctgtcctgaccttacagaggttctcttattgtctcttacactcaataaaatatctttctgatgtggatctaagtgtactcctagtatatcttccgagaatccacaaggatcgtcatagtatagatctactaattcttcaaaggatatttcttccagagcttccttgttaatgtggaacttatcaactaaagcatctagctctaatttctcaattatgctatctaaatcaaacaattatatacacctccttagtaaagtgctttatttagtcctgtaatacctttttacttagtggtattagattttcctttacctgcattctttttctttctatcagccattttggctctaagaacctcaagatcttttcccttaccagcattattctgattttcctgtatttgtaaaagtaatttaaccttttcaagttcaactttcatcacatcagtacttaggccgaagtatacctcaagtctttttagtgcctgaagtctatcctccattttaactgatacgccatctttactttgtttaatctcattgattaaagtaccatctacagccttactagaccttaatagaactagatcatccttgaattggcacacatcagttatatctgcaaaggctattttcatgtactgccttattacatccataccatcgcatagtaattcttcatctctatcggctctgatagcctttagagcttcctgtattttcttcttctttaatagtttagacccatgtgcatgagaattattcccaggataacctgctctagcagctgctgtagttgcattaaagcacttcatgtaatgaaatacaaacaactcttctttctcatcaagatcatacttatcagccagggtcttaatagtcttttttgttttgctactcaatgccacaatatcaccttcttcttctaaaaatgttatgccctgctctttaaactctcttagacactgcctaacaaaggtctgtgataccttagcaaggtttcttagttgtttaggatgtgtaaagggatcagccttcagggcattatatatcaattttttggctttcttcaaatgttcaggagtacagtactctggttcagtgtatgacttatagctcataatacaatatcacccccttaaaatccagactttactacgtgaaaaatggttggcacactaaccttaatgctagtaataccaaccaaatggcaaaattaactatggatttataccactattataccacatctggattaattatgtcaacgttttataattttatttcacctgtcaatattttttcatacatatccacatctattcttccttcctgtagcaggttatcagctgcaatttgtatctcttctggggaatatactggattacctttagtatcaagttctataccagtatatgagtctaccttacctctgttcataccatatccaactgatttatgaacttctagtttttcattatggtcttcttgccagtgttttaattcttcctgatattccttattctcctctttagtttgtttacattcaataggtctattatctttcatcttttgctttagagctgctgtattgggtttacagttcttagatcctccacctgaacctctattcttatcttcctcataagctttattaatctcaatcccaattattagatccatcttctctaccaagtaaagacattcttttactattggattgttaggttgatttttagaaatgatgtcttgacactctttctttaattgatgtggattattacattggctagggcatttttctcctggcccatatggaattgtatatgctaagcagttacctgctggatcccttctataacatcttcttttacatactattttactcatggttaatacctcctaatatattttctttctcttctaataatttttcaagttcctcaagattttcttctttatcactattaccagctttagctatatttagaatagcttctagttgttcctcactcaaaaactcctttaatttctcatcctctaatatattagatacctctttactcatattgttctacctccacatcattacaaattaatttagctattccctcacttaatctgtatttctcaagatataccactttcttaattcctgcattgattattaaattagcacagctctcacatggggataaggttacatacatagtagttccttcagttgagatcccatgtttagcacagtaacttattaagccagcttctgcatggatcacaatatcacatccaggacctaaacaagttttacaatgttctactcctgaaggtactccattatatgaagtagcaactatcctgttatctctaactaatacacaaccaactgcttttcttaggcaagtagatcttcctgtcataagtttagcaacttccatgtaaagtgtttctctgcttattctgttgttattattttccatagtttatcacctcaattttattatatactattccctatcatatgtcaagagaaactttagaaaggtatatcaccataatccagatcaatacattgggctggctttggttttacttttttaggctctggagttttcttgactttatgatactttggagctctggctaaatccttttttaactttctgactctcttcatatcccactcatgtatttcatggtctctaaaatattcattcaatactcttactgcggatctctttgaaggtgtctttacagagcagttattaggagcaagacagcatcctgtctccttatctgatatagtataacatactgtattatgaggggctcctacaggcctatgaatgaataaggttctgcccatataatcaaactcacataatacttccacatatcttttatactgttgtccctggtcattcttacataatacataagtatattctttcatgttaattctcctttctatgttaaaagggagatcatctctccccttaatatctttttattcttctgttgttctcatcaacctcaatcacttcataccttctaaccttatcagatataccttcctcctgtaatactttaggaatatatcctatggcctgtcttttgttatcaacttcaaaatatctggtcaagatcctttttgatgttacaatcactaatcttactttcatattatctacctccatgtggcctgaactacagctccaggtctatgcttagcttcaatcttagcttcttcctcagtatcaaaatagattatatcttccttgtgttcatccttaacagatacccagtgtactcctaaatatttgttatgtgctaatacactaacatcagggttccaatccacatcaactgtaacttgtaaaacgatatatctccttttcatatcagttctcctttttgtatttatttgttgattttattataagagagcctcggaagtttgtcaaagattttctcgaaggaattcgtataatatcttccgagctgagcataatatagactataaaacaaaatcaaggagttgtaataaatgaaagataataatttaataccattaagagatattgccaaagaggttggaataaatgaaaggaaagccagaaagctattaagatcacatgagaataaagcaaatcacaattattattggatgtttacaccaagagagaaaagacatattgtatcagttctaaagagactgcaataggttttctaaaaataagggagggattaaccctcctttttataattttttgagttctggaaaaatccttaattagttcaagtttcgtaaagttctcttgatcttttccattctcttcttaacttggatagcttcttcttcgcaaggagcatggccccctaggaattggtgccatcttctttcaagttctctgtattcagattgaagttccatgaactcaagtgaatgattgtccatactatcacctcctcaacactattataagtgatactgtcatattctgtcaaataaaaaagagagaatgttattctccccatcttaatatctttatagttgctccatcaactcccttgccatccacatcatggacatacttatcaagtctcattgttgagtcctgtataattcttttgtcttctctgtcaaaaaccttaatgacatcagggttacccctgtcaatgatgtaagcaatctcttgagttccatctgcatatgttacttgaagtaatgaatgtagaggaataaagtctggagctgcccaatcaccaatcttaagatcccctcctatactattcttggtctcatatcctgccacatctgtaggctcatctgatgagtaataagtaacttcaactttgaactccattcctttaaatgaatttatcatctcaattagattttgtttatcagttctcagtttatcattctgatattttaatccttctacattgtccatcagtatttcagtctgctcagttaattgtttattcgactcaatatattcttggacagcatttccccaatgattgtttaggctctgtatggttaacagtagccctcctatcacaattattgttagtaatgacataattcttttaatcattctcttttaactcctttatttttaatttgaatttctcaattccagatttatacttacccacaatatcaaaggtatcggttagtattgcataggtttccccatcagaattaaatctgaagcttcctctcttgatgtctcctagcttattaaaggtcttaccctccttgtccagatatcctttatagtccatatagcacagacaagcagtaacaaactcctgcttattcctgaaattatgcttgatacccataccatctacccatttacttaatacaaatagactttcattagtcttctttactttactattctggattagatccttccacacataatcattagcctctttaaatgacttaaatctcttgcctttcagtatcttactactctggatcttggctttataatcctcaaatatacttggccagaagtcttttagatataaatacaaggaaatatcatctaatttagcattcggatcgttaatctggattacaggatgaccatccattgctctgatattattccttagttgggtattctctctcttcattttagatacttcaatatataatttaacgaatgcgtcagacaattcatgattggttaattccctttttaggggcttaccatctttactttctttagtagttacaatattaaagtagtcttgtaacctatcccagttattcttcattagatctacctcctatgcttacattatacatatattgtactgatatgtcaaagtccaggcattaactgatatctgatatgcctatatttttaccccatatcagtctgatatcccacatatcagttgaaactacaaaatcacaaaggcattggtatcactggcgtagagggatatcagttatgccccctttatatatacatagtattatatatactatataataatatattattatatatagtatatatatattacatggtgattacatcaatggcaggctattgccttgcctccattatcattacggcaggcatatccatgcttccgagcttttgccctatatagaaaaacccagacggtcagcgatcgagctcttgattttgttttgtcgagggagagaacagtaagagagaacccccgaacgttgacagttgtacttacttctcttataatgacagtaaaggagggataaccatgaaaacattatttactgatacaaaactagtattaattgaaactactaacttcttcattatgttacaagaagaaggtaagtatgtactatctaaaacaatcgataaggagatgggagaacaaatacacagagtatctaagttagctgcccttgtatatactaatgaggagtatactaactctaatgaaccaagatctatatacttagatgacaatttcttatacgaagtgcttggtaatgggaagtatattataagatacagtatataagagcccacaatcaattctaaggccttttagatatgtggtaatgtgattttacttataatgtggtagagacaccttacaggagctgctagaggcctttaaaggaggtatatcatgtatttatgtaatggtaaaatagtcaagaataaaaatgacttaaaagataagtttggtggtaaatcagtagtattcatcgatggggatgtagctacagtaatggactttagtgacagaaagccaaagataacaaaatatcttattagggaggtatcacatgataaacacatcattattgaagagactggaagggatagaggaaaagcataagcaaaatactgatgagataagaaagaacctaaactatgccagatatttgattgagaaacagtattgtcatttaacaaaagaacagaagataaaattgggacagttcttaggattgactgagaagaagttaaaagaaatacaagagataaataatcagttaataaatttgagagtggggctaagttatgaagtcgtatgtaataaccagaaaaaatagtggggtatctttagcagatacagacatgggacaagtattagctaagatactatgtaagcatgggggaacacttaccattgaggaaattgaaccagaacatattggtcaaactttttctattgtagaaggtaaaagaatatggtataatagaaaaggaggtgataatattggggagaagaagtgctatgttaattctcaagtatgactgcgaagaaactccagaaaggattgaattacgaaagaagtggttacagatttgtcttcattcaataatatattatagatatgacaacaatatctggacagaccaacaatgggatgagactgccagagaggtagttaaacttaagaatgagaatccaggtttagtaaacagtatgccatttaggaatgaccttaaagtctttgatggatccactggctttaacctttcatgtatgcaagatattaagatgttaaggtgggctcaaaacttacttgactttcatgttaaacgaggacttgatggaaagagtaagaaaaagaagaagaagaggaggaaaaagaaatgaacctacttgagcactatataaaaaaggtacacagtgtaagagagtaccatgaatttgataatgaaccttgggctaaaggtaaacaatatgtagaagtagacatggactatatttgttattctaatacaccacaaagagtgaagatggtatttactgttgatgagtgggagaagataaaatatagaggctactacatgggataggaggaatagttatgataagagaaatgggcatgagaatgctaataccagaaatacatgatataaaagatagggatatacaaaattttgtaagaaaggccctaaatgagatagttgatgaaaagttctttataatacctgcaagtagtactgggaaatatcatccaacttatagtgcaggggtaggaggtttgttaagacatactaaagctgcttgttatataggtaaagcattatgcgaagctgagatgatatgttcaagggacagagatatgataatagctgctttaatattacatgacattaataagccagataaagaacatccatatatggttagagagacactatcacccctagaggaagagtttccaataatatacaaagtggtagttgaactaattgagtctcatcatggtcaatggggtagtgttcctattaatagttattcccagagaatagtacacttggctgattatatcagttcacagaaaggtttaatattctcatatgaccaaggaactgattattctgacctgttatgggaggagaagtaaatggtgctaggggtaataaccctagtatcaatatttttactaggagtgtttataggttttgaggtgaagaaatggaactaggttttgcgatactagctataatagtatcaatatttttagaaactaaatatataaaggagtagattattatgtcaagagcaagagctgcaaggagaagagccgaaagagagaacaaaaatcttaatgttcttaaagctgtggacatcatgttagccttatcatgctatacattaaagaaggaaggttatggtaagactagaatgactaggtttgtggaagggatgagtaaacacacagaggagattgaaaagggaacacttaactatgaaaccataatgggagagattaaggatttagtaccaccaggtatatttgatttaggggaggagtcaaaggagtgatagtattgggatatttattatgggcatttagaatattaggcatacttgtaatagtatggtgtataatggaggcgatcagttgtgagcaataagttatattttaggtatagtgctatgaactctggaaagactactcagttaatccaggtagcacataactatgaagaaaggggaatgaagccattagtagttaagcccggaattgatactaaaggtggaccatgtataatcagtagaataggggtagcaagaaaggtggatgttcttctacctcctagagttaaattatcaaaaatactttctgactttgagtctaattattgggcagtagatgttatattaattgatgaggtacaattcttatccagagaacaggttgatgatctgttaaatttatcattacattatcctattatatgttatggattgagaactgactttaaaagggaaggatttgaaggaagtaccagattattacaagtggcccataatattgaagaattaaagaacatttgtcaatgtggtaaaaaagccacattctcaatattaaaataccagggtaaatatactgaccagggtaaccagatacaaattgataaccagcccgaaagtgttgaatatgaagccgtttgtaatgaatgttataataaattaattttttctaaataactcgttgacaggctatataggatatgatattatagtattgtaatcaaattacaaacaccaaccaaaactttataattagttaatttcaaactatactaaatttgttatttaaaaattaaaaatatggaggaatgattattatggcaaaaggaaaagcaaaatggttagaggaagcaaacaataaggagctaattgtaatcgtacaatctgctttaaattctggagatgagaaagaagttaaaaaggctttaaaagctattgtggaattagatgaaagaactcctgacacagatggacaaataactgtagaggaagcattagaatcattagaaatggctgtaggaactgtaaaggctgcataccaagcagaaatagatgctgtggaagatgaaggtgtagtagatgctgacttcgaagaagttgatgaagacgaagcagaagaagaagatgaaaatgatttagaatcattatctaaaaaggaattagctgctatggctaaagacttaggtatcaaaggagctaagaaaaaagataaagatgagttaatcgctttaatcaaagaagctcaaggtgaagaagaagacgaagaggaagaagaagaggatgaaactcctgactactctgaaatgactaagaaagacttaattgctcttgctaaagaaagaggaataaaagttaataagaaaatgaaaccagctgagataattgaattattagaagctgatgatgaagaataattctcatcaaataataaggggagcaaacttgctcctcaaattttttacttattttagaaacagatgttagagggggatgtataaatggcaagaggtggaaattcaacttatactaaagcagtatattgttacaacaataatagggagtatagatccttcagatatgcagctaaacagttaggagtatcggctgttagtataatgagagtagttaacgggactaaaccacatatagggggattagtattcgctgagatagaggaaggcactagaaaattaaagccaagaggagaagtagttccatacttgaaagaattaggttgggataatatagacttataatagggggtataatatatggacataaagttcttgaaggatatattctctaaacaatgtgaaaatagagattacattatcctagcagctagaaaaggtaaagaatggaaagatgtaccaatcaaatataataagaataacattgacaaaaaactaaaggactttgaacaacagtataagggttatgatttatattggagcccaatgccctatagtaatcctcaaagaaggatagttaacttcatagagactaaatacttaatacaagatatagatgagcatactgacccattggggattaaacctaaaccaagttatctgtgggaaagttctcctggaaaatatcaggggctatgggaaatggataggtatatagaggctaatcaatatgacgaaataaatccagcattagctaaacatataggctgtgactcctgctttgatgttactcatgtatatagaataccaggaactattaactataaatacaagaataaaccaaaagtaaaaagacctatacacactaaggagatatataagcctaaggtgatcgctaaggctgttaaggctgtaagtaaatctaatgatagtgttaaggtcaatataggaggatctgaggcctcacaatctgaaagaaagatatatgctaaatataatataccaaagaaggttagagacttactggctttagatgacattacttctttagatagaagttctactatatggtatattgagaataaattacatgaaataggactagagcctaatgagattatattattagttaagggctcagcttttaataaatataagggaagaaaagatgaagaaacaaggttaagaaaagaattggataaaatcataggaggagaaatagaggctgatattgaaaaggctgaaagtactaaactgagaatagatagttatcaggatgttatgggtaataatggtgccttcccaggttggttagtacaaggtttctggggtagaagatctcatggaattgtggctggacaaccaaaggtatttaaatccacatttacacaggacttagctatatcagttgctagtggaagacccttcctaggtcaatatcctgttctagaaccaggcccagtaattgtagttcaaaatgagaatgctgactggattatgagggatagaactgaaaagataattagccacagaggagtagttggtaatgtggatataaagggtaagagaagacttaaagttaggtttgctccagatcttcctatcacttttattaatcaacagggatttatgttagatgaagaatcccatagaaaacagatagaagaattaattgatgagataaaacctgtactagtaatattcgacccattatatcttatgtttaggggagatcttaataatgcagctgatcttaatcctgtactacaatggtgtcttaaacttaagaatgagaagcatacaggagttatgttaatacaccactataataaaggtggaaatgccactcaaaccagaggtggtcaaaagatggctggttcattcatattacatggttgggtagaatcagcattatatttaaaaagacctgatgacttagaaggtgacgatgaggagattgaagtagatatagataaccttgataaacaaagccatttaccaagtaaaatcattatggatagagagttccgtcttgcaggacaattccctcaaattgaattgaatttatcaatgggagaatttggagatccatattatcatgtagaagtagcaatacccagaaaagaagtaattgtgaaacctgaggacaaagccaaagttatagaggctgtaaaatcaggagctcataccaaggaggagatagtgtcaatatcaggattaaattcacagaaggttaatccagttctagatactttaaaagatactattgtatattctccggataaaggttataatataagtaagaaactaaatattgggaggaaaaaggcatgataataaagtgtaagaggccagcaggtcataatcatataaaggcctttgtagtagtaattattgctagaggtaagaagaataaaatcacttatcattcaggattgaaatatttctatacctataaatcagctaaattatttatagacaaagttatggaagaatgtccctgggctgaattttattgggtggatgtccatgaagcccataagatccctgaaggcgaagagatacctaagaagaaaatgtggtgtccatattgtcaaactattcaagaatttaagagaagccaaggaggttacaagaattgccctatctgtggtataagtgaccaagacttttatgtaaaatgtatgaatataagatatagggaggctaaggctaatgcgaagaagaaacttgaaggaagtaatactaatcctagggatatcattgtcaatggggataatgctaactcagggggcaaaactaatagaaagtcatcaccaaagaaaaagtcaagaaaagttagtagaaaagcttcataatgctttagactataatgttattgagacttctccatctggactagatggggaggatcttattatcaaactaaaccttaatagtcctaaagaccttacccctaacaacttatctaagttagctaatgaggttatggtcaataacttaggagctcagaattatactatacttgtttatgatagtaatagaccagaaaatcttctggctgttatagatatacctaaaaattctaaaataacctttgacataataaattaattatggtaatataaaaatgtagaaggaggagaatttaatggtcaataaaaagtattacatcttgaaagaccttaatgatgacaaaccccaactatggaagggaagtttaaccactgctactaagatagcaggagcattaggagttagtgtgataaaactaaataggtatttagtaagaaagggatttgccagaaggtacaatgagcatacacttgagataatagacccaatccttgctaaagaacttggttattatgtaactccaagtaagtcccttataaatcctttatttgaatataatgataaaggagtacaatatatactaaacttaatagtagaagatctaaagaatggaggagagctttaatgattatcattttaggaatggataactcaggtaagaccacaacagctaagaacctaactaaacacagaggaggagaatatatccaatcaatgggacctggttcttatgaagaacaaagagaatgggtattaactcaaattgtgagaaaaggtgaaagggaagctatacatgatagatttacttgctttgaagaaatggtgtatggacctatcatcagagatagtagtaatttcaaccttgacagtaaggagctaaagatcttaaaacatctatgtaagccaactattgtatatgctagaccacctagggaagtgatcttcaattttggtgatagagaacagatgccaggagtaattgaaagagctgaacatctactggctagatatgatgaactgatatggaagttattctgtgatggatggaatgtactggtatatgattatactacttccaatgtggagaagctatcccagttaatagatgactcaagtgctaaagaagctataaaccaatttataaatatatcaagataagaggagagattgttatgaatataaaccatgcagtagaagaaaaaatagaaggagatagattacaagctatctttaatagacaaaaggagttaatggagaaatatcatcatatagaagctagatcaggattatgccaaactgaagactgtccagttaacttaaatgataaaagaggtcaagctagacttaaagattttgcttggagaatgactgaagaagtaggagaagcattggatgcttataatcatgaagaccattaccaagaagaattaattgatggattacacttcttaactgaatttacaattctagctggtaaggattataatactatagataataatgctatattagttgatagcctagagaacttatatcataaggctactacatcaccagaatttcctgaaatgttagtagaagaagctgtaactgacctggtaagagaaatgggtatgtgctgtaactgccttaagaataaaccttggaaacaaacttcaatgctaacagatgtaaatgcttttaatcaaagattattcaatgtatgggtatgttacattaaattattagctgtatctggcttagaggtagatgacatagtaaatatataccttaagaaatcacaggtaaataaattccgccaaagatctaattactaaaataaatacttaggagaaggtaatatgctaataagagactataatgattttgatgacttattcttaaaccttaatagggaaatgattaccaatccagaagaaactatgatgtatactcagaacatacagggctttcaggaggacttagttctctcctgtaagtcccataaatgtactttaaatctaggggactttggatataaagaaggtaagtggggacacctattaagatcatacattgattatccacaattaattgaatttagagaaaagcttaccaagataagtggtatgagctatacttattatttcaacaggaaaaaagctactaatggttcttgcttgatagctgcagtagtaactagaccaaaaagaaaaggaccttggaaacacttaaaaattatgtatagagtatgtgaattacaaaagaaattcgcagctgatctagtattaataaacaggttcattgaagaactacctcaagaagtatgtgagatagataatattacttttcatatgtctcaagcttatttgtcaggaatgtttataaatggatatttcaattattttaaggtaccaagaaagagtattgctaatagcaaacatccttggcataaatccttgaatagtaactataacaggttctttaaatcagaggaccagatacactcttataaagctctccagaagatgcagttattacattttggtctggagaaatttccaaagatagatatcaataaattatctattgacaagtactttaataagtagtataattaacttaacaaaattaaataaatggaggaattaaactatgagaatttatattaatgctcaagaagcatttgaagaagtaaaaagagatttatgtgaaatggggattggggtaagacccaaaactatgcaagataaagttatagaaggtaatccagattatttcacaaaggagttacaaaactatagttacacaattctagaaagtaaacctgaagaagttccaggtgtatctcaaccttgggcagatgctgaatttagagaaaggatctacgatccacaaggtgtcatcaatcaatactctcttgaagaaagagaagaattatttggtatacatccacatcatactagggaggctttcataaatcctggtaaagcttatcaattaagacctgaggtatggaatgaatatctaagagatggaaaatttgggtattcttacaatgaaagaatttggcaatacagacaaattgaggatatcatcaatagaattaaagaagatccaggctcaagacaattatggttatctctgtggaatccagctattgatccattcaatataggaggagtaactagagtaccatgttcattaggatataacttccaagtaagagaaggtaagctaaatatccattatgttatgagaagttctgattttgctactcactttgctaatgatgtttatcttgctatgaaactattacattgggtagctgaacaaactggctatgaaccaggaagtttctctcatacaattttctctcttcatgtttacaacaaagatattaagggggtattctaataaatgagttacatgagaaaagaaagatataaacattctgatcttaataataaggttaacaagagggaaaccctaaagcaatttattaggaatactgaaaaggaatttgatttagaaccagctaaccttggggacatgactaggaatgaacttaataactatataaattatatggatgaactgtggagtaagtaatatgtataattatagtgatgataacagacctaagaacaataacaatggctgtcttggttgtttaattataatcttagcagctataggattatgggtaataatttttgatattgccaatataatatatcatatgatattctaaatttaaagggggctatcctaatgaaaaatataatttgtcctatgtgtaaaaactcagtaacattaaaaagaaaatatggagctatgttttggatcatgattttcttaactggaggcctatgggtagtaaccatacccttcaaaaaacataaggtctgtccagtatgtaactcaatcataaaataaagataagggcctttaggggtcctttctatttaggaggtaatattttaaatgagatgtaacaactgtaacctatatactcactcagctccctcatgtatagaaggaacttgtgtaggaaagaaaaagaagccaagaataatggtcataaatagtttagctaatgatagggatgaggccaatagaatagctactcctgataaatcattacttgataaaatggaaggtctagacttttattataccaatgctattaagtgtagaactcctaagggtactaaaatcaaagtatcagagattaagaaatgccaagaacatttacttaaggaaattgaaaaatataaacccgaatatgttatgatcttaggatctcaagcattaaagatgctaagtaatgaaggtataacttcaatatgtggagtacctaagaagcatgagaaatatggctttaagtttattgccagctattcacccggtgtagttgcatatgacccaactaaagcacaatttgtagatcaggcctttaataactttaaagccatggtaaaaggtaaagagcatgaattacctgatcttaacataaaacttattactagtatgaaagaactaaaccaggctttcaaatatttaagggatgagggttataatagagtatcatatgatatagaaactagaggcttagataggtttaataataacattactctatttggttttggtaatacccaagtacagtatatactgcctttagaagtcaaatatagcccattaaggggtaagcccatagcacaaagaagattagctaaatccttgattaaaagacttaattctgagatgaaggaaagaatagcccagaatggtaagtttgatgataatttcttaaaggagaaatatggtattaagccaatcataacctttgatactttactagcctcacattgtttagatgagaatactcctaatggtcttaaggagaatgctttattacattgtaatgctaaagactgggatataaataagaaattaaagactggaaatgtggagactaaatcagactttgaggattatgttaggtatctggggtatgatatatactatacatttgctctatataaaatatttaataaaagacttaaaagggatgagagcttatataaactattccaccacttatacatcccagctagtaaagcttatgaggatgttcagttcaagggtatatatgtaaatcaggagaaattcaaagaggttgaaaaatacttaagatctgaactagataagattgagactggacttaagaagtatactaatggccaggatattaactggagctcacctaaacaggttggagaatttttatatgatatacttggtcttcctgtgattgaggttactgactctggagcaccagctactggagaaagtgtattattaagactaagagataaacatccagcagtagaactactattacagcataggggagttcatatacaaatttcccactttatagatggttggctaaataggatgcacaatcatagattatatccaaactttaaacttcatggaactgtaacaggaagaacctcaagtaataatcctaatctacagcaagttcctagagataagaaaatcaggagtttattaggaccatctcctggaagagtattcattgaagccgatctatcccaggccgaacttagaatagctgctatgatggccgatgaggataatatgaagtttatttaccagactggtggagatatacatgactccacatataatattatatctggggaagatatcaatgatgagaaagatccagcagttaagaaggagaaaaggaaaaaggctaaggctgtaaactttggtttcttatatggtatgcaatggaaaaaattcaaggattatggaagagacaactatggtcttaaattaacagatgaggaagccaaaacatatagaaggaacttctttaataaataccctaaactattaacatggcatgataaacaaagaaaaattgttaaagccaatggtgaagtaagatctctaataggaagaattagaagattacccgatatatattcatctgatagatctaaagctgctgaagccgaaagacaatgtattaactcaccagttcaaggttttggttcagatatcactttattaggcctatgtgagattacaggctatgctaaatatgttaatcctgaatatgtattagataagtctaagtttgatgtattaggctcagtacatgactcaatattatttgaagtagataaagactatgtggaagaattagcttggaaagtaaaatcaatagttgaaaataataaagtattaaagaaagtatttaaatttaccccaacagtcccaataatcatggatatatcagttggttattcttggggaggatgtgttgaactggattttaaaggtgattggaaaagccagataagaaaagtgttgacagatgaataattatctgataatataaatattgtaatgaaaaggaggtataaggatgttaaaaataagtaattccagaattaacaaattcttgtcttgtccttatgcccattatgttaaatactatgaaggtctggtacctaaaagaagtggagctgccttacaaaggggctctgctatccaccaggctatagaagactaccataatgggaagagttggaaaaaatctgttgataaattttccaaagagttttacaaaaatacatttaaagaagagatccttgaatttggagatattccaaaaatggtttattctttatgtgataactatttccactattatgatgaaaaagaagataatgtaacctatgtggaaaatgaacatcacttcgaattaaaactatgtaagggtgtaactctagaaggctatattgatagtgtcttagatgtggatggaaagatatgggctaaggaaactaaaacctacaaaaagatgcctgatagaaatttcctgatcttcaatagacaatctgctatatatacctgggctcttctacatgaatacccaaaagtaagtggtactatatgggatataatattagctcagcaaccaggtagaccagaattaactcaaaaaggggtattatctcaaaagaggattaaatccacacccctagagttagaaagaggaataagagaattaggattagatcctaaagattatgagtcttatattaattctgctagatgggaagacttctttgtaagacacccaataatattatcaaagaatatacttaacagtgtaatgattgatactattgagatagctaaacttattagagatgagggccacaaaagaaaggaaaagaaccttggaaaaggttgctctttctgtgaatataaatctttatgccaagctgaacttttaaatcttgataaagaatttattattaaggctgactacaaacaaagggaggaaagtgacaatggcaaaaaagcaaaaatcaaaatcaaatagttttgaggacagattagtggatctatatgatatagatgagcccacaatactaacactttatggaagatctggttcaggtaaaactactatctcaggaacactacccaaaccaatattctttattgatgtaaaggacaaaggtactctatcagctagaaacaagcttagagttaaaagaggagatatacaagtatttagtctaaagagttttgatgacatatacgaggcttatgattacctatcagaaaacactgataaatttaaaacagtagttatagaccatttaactgctttacaagaattaggtaatgaaaaggtcaaagctgaagaaggtaaggaccagatgagccaaagaatgtttggaaatgtggctaattatatgaaagaggttataaacctttataaagaattaaatgaggaaggtatactaccatgctttatagtacaagataggttagaatctggtgatggtgaaggagaagaccaattaatgcctgaggtaggaccaggattaatgccatctgtatctaaatatttatgtgctgtatcaagagtaataggtcatacttatttatatgaacactcagaaaaagagggtatgaaggttaagaaagaaatccagtatagactaagactaggacctaacccttattatattactaaatttactagacctcaaggatctgaatgtccagcttatctggtacatgatttaaaatcaccaacaactatctgggaggatattgaaactattctggctggtgaatggaataataagccagctaaatctggtaaaaaaaccagtaagaaatctggtaaaaagaaaaaataaaattttctaaaaatacctttgacaaccaattaaaaatctgataatataaacttgtaaacaaagaggtacaatatcttgacaaatatttatctcataatgatattttaaaatttaaggaggacaataacatggctaaaaagactactaagagaggtaacaaaaacaaaggaggattaaagattgatctttcaaacgttgaaacttcagttactatcccagaaggaaattacattgtggaagtagaagatgtagaggttaaggtttctgaaaatagtggaagcaattatttatcatttacttttgtaatagcagaaggaaagatgaaaggacaaaagttataccacatttgctcacttcaaccacaagctttatttaacttaaaaggtgtgttagttgctttaggatttgatatccctgatgaggagttcgaattagatacagaagctctagttggtttacaatgtggggtagaagtatcacatgaaatatatgagggtaagaagaaatcaagaataactgattttataaaccttgacgaagctgactctgatgatgacgaagatgaggatgatgactcagatgatgatgaagaagatgatgaagacgatgagtctgaagttgatcttgaagaattagacaaggatgagctaaaagaattagctaaggctttaaaaatcccagctaagaaaatcaagaaggctaaaactgaagaagatctaattgatctaattgaagaagaagctgacgaagaagaaatagctgaacaatataatgacctattcggagactctgatgaagatgacgaagaagatgaggatgaagaagaggaagatgaagaagaggaagatgaagaagaaaatgactatgagtcaatgactttaaaagaacttaaagctgaagctaaggacagaggcttaaaggttaaaaaaggaatgtctaaggatgacatcatagaaatgctagaagaagatgatgaagaataaaatttaattattaaaatatgagggcctttaaggtcctcctttatttacccttggaggctactattatgcttgaaagagatgtggttaaatccataatgaatatgcttaaaaaagaatacccaggtttttggtttaaaactcatgggggaccatttcaaatagctggcttacctgatatactaggttgccacaaaggtaagtttattggtattgaagttaaacttcctggaaaagaaaagaacctaactcaaaaacaaaaagacattataaataaaataaatctagcaggaggaatagcttttatggctacctcagctgaatatacaaggaggagattacatgaaaaatttagaaagacaccaacaattcctaggagaactaggagatctgtatgaattaaagaataatctatatggggataatttccacaagacttatcttgaatatggaaaccctgttctatgtataagacttgaagataagctaggaagagctaaaagtttattactaggagatcaagatgacttcccttcatatgctgctcaaaaagaatctgtggttgatactttactagacctagctaactatgccattatggctgctatggaactaactagtgatgataactcagaaatacatgatcttagtaaagaagaatatgatgaagaagacctagatgataatgacgatgatgacttagatgatgatgacaatgtttacgacgaagaagaattagattttgatagtatgaataaagaatccttaaaacaatatctaaaagataatggggttaaattccatagtaaggcctcaagagatgaacttgtaaaactggctaaggaggtataaggaggaggctttaatgcctcttcttttttagtatgaagagaaaattatttaaacatcagaaagaagcattacaactatttttaaataaagaaaagtttgccctatttatggacatgggtacgggtaagaccttagtccctattgtggcccttgagaaacttgaaggtctagatactgtactaatattctcacctaaatctattgtatttaactgggagtctgagatccataaatttactaaacttaaggaatataggatatttaaattacagggtaataagaccaaggttatggaaacctatagagctataaaatcctactcaggattaaagattattattgccaattttgagaaggctaggttgatggataaataccttatgaacttaaagccacagtttattgttgttgacgaatcccataaggtaaagaatagaaatgcccagatatctaaggctctatataaaattgctactaaatgtaaatataggttgataatgtcagggactcccactcctaatggttatgaagatttatttatgcaatataaaattatgaactcaaatattctaggagttaattggaaacagtttgaagatgactttataatcaaaggaggttatatgaactatgaaattgtggggtataagaatgaggaaatattaaagaaccttatgcaccagaattgctatatagtaagaatagaagattgtattgatttaccagaacaacttcctgatctgtatttaacctgtgaattaaatagtaaagccagaaaggcctataatgaccttagaaaggaaatgatagcacaactagatatagtacaggaaaacattcctagaaagcaattaaaggccttattaaggtctaatggtataccctatgagagtaatgagccctatgaggatttattcttaagggctaatatgtttatcaaccaattaacagctgatcttactattacccaatatttgaggctacagcagatctcaggaggatttatcacaaacaatgtaggaaataatattaatattgataaaggcaaattaggcttgttacaggactatctagaaggatataaaaagcctgttgttgtaatatgtaattttcttgaggaaataaaacttatacatgatacttttaaaaagacccacagagtagaatgcttaacaggatctactaagaatagagctgagatcaataaggattttcaggagggcaagattgatatattaatactacaaataagctcaggtagtgttggtctaaacctcttcagggcctcaaggttaatattctatagttggaactataaatatgatgattatgtgcaagctattgccagaatcaaaaggaatggtcaaaaggagccttggcaaataatacacttaataacggagaatactattgatgagaaaatattaaaatcaatacagcttaaaagggatagagcagaaaaactgttgactattgataagtaatgtggtaatatagaattgaggtgataagtaatgagaaaagaacaacctagaataagtaatcatactgaaatagctaaggctttaattgaggctggtaaaactattaaagctctaaccaagattaaagtcaaggaggaaaagaaaaaacaaaaaagacttgaaaggttaagactcctaaatgaggaaaagaagaaggagagagaattaatgaaagaatttaatcccgatgagcctaagaagccaagaaagaaaaaggacaaacctataaagaaggttgatctgaataaagttgaggctaagggaacttaccctacaccttctggaggtaatgcacctacgggaacagttgacttaaaaattttatgtgagtcattaggattagatccaagtaaagccagggccaagctaagaaagcaaggtgtaaacaaaccctataaatggtcaggatctgaacttgaggatattaagaaaatgttaaaataagggggaggtttaaaaacctcttctttttcgttgacaatatccacagtatatggtaatataaatattgtaatcaaacaaaaaaggagagaactgaatatgaaagatcttgaaaaacttacaagggaagaattgattgaacttgtaaaggagttatctattgattggacaggagcctataatagaaactataagattgaccttgatgagtatgagattgtatatattgatcttaatgatctaaaagagttcaatgataaattaggtcatctagaaggagatgtgtatatacaatacacggtaaatcttattaaggcccatttacatcctgagaaggatatattgattagagggggtggtgatgagtttgtagttatcagtgatatagcttataatctgtgcaataccttgaatatataccctgagctatcatgtggctatggtaaaggtaaaactattgaagaagctatagtacaggccgactcaatgatgtataagaataaaaaatctaagaagttaagatactcaaaggaggattagttattatgaggttattatggttaaaagaatatttggatatatgcaatatcttgggtattgagcccacaatggaatcttgtgctaggtggggaaagaataaaaaactatcagggttttcattaaccccagtgggagcaactaaatagttgcttctttttaaagcgatccgatacctagcaactttcatgccaaaaagaaattcgggattttctttgacatagactccagagtctggtataataatcttgtaaacaaaattaattcaaaggagttgttaattatgaataacaaaaaatttcaagaaactttagaacaattaaaggaggaactagaaatacaaggggtagaatttaatgatgagaatgacttaatagctgctgttgaatacatcatagaatatgattaccacccagaacaatatgtggaagatactttatgtaactaccctgaaatgttcaaggatctataaaactaaggaggtgtaaaaacctccttttttatttttctaaaaatctggatttaatcgttgacaggatcgggactatctagtataataatattgtaatcaaaattaattgaaggagatgttaactatggaactaacaagatcagaaaaacttaatgtaataaaaggaattgctcaaaaggctatggataataaaatctatccacaatttagaaaagaactagataaacaggtaaaatcctttggactaagcaacaaagttagggaaagtgaattaggagactacctttcttgctgtatggttgcctatgaagaggttatactaaaaatgaaaaaagccaattaatatgggtggccaaaaggccatctatttttttcgaaaaaatctccagaatctcgttgacatagtctgggccctctggtataataataatattgtaatcaatattaattaattcttaggaggaatgaaaaatgactaaattagaaatgttaaatgagatagaaaaaataaataaggtggtttttgaaaagaacttccaaaaacaattcttggataaggtgatagaactactacaacaaatgggagtaactaaatattatgtatgtaaacatcataaaaaagctgagattgaaaaacatcttgaggcttgcatctgtgcaatatatgatataggaagaagggatgatctaggatggtaaaccccatcctttttcttcgaagtttttcgttgacagatccagagttctctcttataattaaatcataaattaactattggaggtaaacaaaatgagagatatgatagaaaatcaattagctgaatatgaggtaaaggagttatacaatgaggccacaatgatcttaggaaaagcatttggtgtaagtgctgttgatctttatatagaatctgatgtggatgctaactactatggtctatgccatagatcaggtaataaatttactgggattacaattaaccttttccctttcaggtttgcacaggaaggagaaaaagcttatgataaaatcaaaaaatttggctgggatattaaggactgtgttcttgaaactatatgccatgaattggctcacttaacttattggtcacatagtcctttacataaaaaattaactagtctttattacaacaaagtgcaacaggctagaaaaggtgaaaactcagctgtagcacaaactagaagtgatatatacactttaaaagatttatgtgaattaatagaactagatccaagaaaggctagaagtatattaagaaagaataatattgagaaacctggtaaacagtgggagtgggagcaaggtatgcctaaagatatatatgatctattaatcaacttaaaggttaggggaagaaggtaaacttcttctcttttttcgttgacatatctcgagagtgctggtataattatattaacaaataacttagggggtaaatcacatgatagatatatattatagtattcaagtagaagctgaaaacttctttggttgtcaaaaagaagatggaagctgggtagcaacaggagcatttagtatacctgttaatagcataacttttgaagaggctgatcaattatccaatgaggccatagatgggtggttaaaggagtatgaggttactaaggtaataagtaggagatcacatacacaggttaaattagattggtataatagttatatcaaggatgatccattaaagggtgatataattaatatggtgtaccctgatctttcagataaagctaaaatcaaatatggctttggtaagatatgggctagcactatgtcaaaggttgctaagaagggtttacttaaaacttgccctagatgtggaggcactggccattactcaagaacctcagatggtaacactacttgctttaaatgtaagggctttaaatatgtgataccaactaagatctcaaagaaattttataaatctgtggagaaaacctttgacatctctggcaataactcttataataaacttgtaaacaaaaacaaagaggagatgttaaatatgaacttaactgcaatggaaacaaagatattaaatgctatgagaaagaatgaatttgatgatggactagatgttgactgtgtatgggtattctcagtaatagaaaactcaggtatagaaggaactaaggctagaggtgtgatctcatcacttgttaaaaaaggtttagtatttgctgatggagaggtaataggttacacagaagaaggaagaaaggtctttgataatgctgatggagaagaatgtaactggggaggtccaaaattattaaaagaaatccctgacaaaccagaggaaatctcttataatgaaaatgtagataaaacaaataagaaagaagaggtaaatgatatgaaagatttaaatactatgaaagctgttgaaattaaagaattagcaaaggaattaaaagttaaaaactggtggactatgaaaaaggctgatctaatagctgctatccaacaaatccaacaaccacaagaagaaaaagttgaagaggtacaacaaccagctgaacctgaagaaaaggctgaacaaactaaaattactcttgatctaacagatgttaaggaacctgaagaagaaaaggttgaaactaagaaaaaaccaaaaactaaagaaggtgtatttacactaaagatgatacttgaagaattaaatatgaatggtaaaaaggcaagaaggatcttaagaaacaaagaggttgtaaaaccaggaaagcaatgggaatgggataatgaagaagaatttaaaaaggttaaggacctactttctaaataaagtaggcccaacctctatcccctattgatttacaggaggatctgattttctcttatccattaactgcttccatacttgattaccaaaggaagctacagctgcacatattaaaccctgtataaagccattcaaaaaggtcttggctgtaaaacctaattctaattgaattgccatatataagattgataatgatatactgaatatcaaaagtattaatggtatagaccaatctggtatataaggcttagccttgataaacagacctaaacagtaacatgatacaatgattattaaaagctgtggatcaatgtaattgaatattaagtttactaaattttcttccatgataaataccccctaaattatctctacatattttgaacttacataaccttgcttcttaccgtggctagtattatattctatatgataccaaccattcttacttcccaatatagtaactctctcattactaaatactgagcctattatattaccattcacatcatctcttacattaagagaagtgttaactttaactattccttgtttaacatcctcatagaatttctggctttgctcaccctcgtagcgaacgtatccatcagatggagtaccatcctttctataaaatgttattcttaaccagccattagttctatacattgggctagccttttgaccaggctgtagttcttcattatgatctttgatgttaacgtcttcagggttccaccacacataagttactccattgtcattttgatatttcatgtggtagtcaaaacttaatctgctgtaatgttttatgtcaatataagcatggtacttcttattctttccaggatatacaacttctatgaaatttctagaaggatatattccgagaacaaataaattatctaggctatcaataaatctaccagggactggcttacaatcctcatctagaacttctattgaaccttcccccactaaagtagcattagttcttgtctcattagactcatagaatcctttggggttattgattactggtgagcttgagctctctcctgaatttactctttctaggaatgtattccagtaaccattggctatcattcttctaggacaattttttctactggcatcatagtgtcttactactttacaattagaatagtagccattctttaggtatctaactagctctacagcattatcaactgccttattgtagtcagagtcaggattaacacatatttctatagatattgtatttctattattgataccgtatctattatgaccatctccacaattccaagtggcgtgtttgtgttctacagcttgatatacccctgtatcatcgacataataatggacactggctttacctatatttccatttgcttgagccttacagtgggtttcggctccagcaccccaagaggtattatcagtttcgtggataattatatacccaggattatttgcatttagagtaacattcgtagtacttaatcttttattgattttcataataaacatctcctttatatattatagtgttttattgggcctgagaggctcgctacagcattttaaccacctccttaatatatttccttatataaaacctaacaggccttaaatggcctgctaggcttataagttaacctttgttactaaataggtgatcttttatagtatctacatcctctttgatatcctcaactacattgaatttatcaactagcttatctatcacttgatttaatttattctccctttctctagcttcttgtctagtgtcatataatagccatacaaatagactacaaaagataccttggctaagaacttgagttagtatttctttttccatagattacaccctttccttaaagtcttcaccacatattcttttatagtcctctggtgtaatttctccttccggattagaagagcattttaccgcctgatgtaatttgtccttacctattgctccaattctataagccatttcccagaaattcataatccctacctccttatttattcatcattttaatctttatatcagctagttcttgtgttaatactttcattatggccttagtttgcattagctctaatttagtatcagcaagagcctgggcttgataaccaattaatttattaatatccagaggattaggatctatagcctcataggaagtaaataggtccttatctttgatactgtatagatctgatctctttttactaatatcaaatttggttgggccaccctttatgtggtcaaataaacttacagtcatttgtatggctgaaagattgtctagatcaattacctcagtgttatccacaaaggctaaatgcccttgtgaattatgaggtatatggagacatataatatcttctatattatttaatatttcactatcctctctatagtatagaggttcaggcctattaattaggtctaatatcttagtaacttcttcatggtctttatctataaatgattttacatcttctgagtcttctgcctgatttatcagcatttctttttcatcatcatagaatataaggtctatgattttattagtttccacagaataattaaatcctactattctcatgttttatcaactcctttactcagtggctaaataggttagtattatttgagttggcttaccagctaccatttgataacatccaccattcaaatatgagttattccaatagtcaatagtacaataacctgaggtattattagaagcgtcattatagttatgtgatactagagatataggtaatacccaattccaagccttaggaaaatgtatagtataacttacacctccacctgagttagcataacccgtcttaactatttgacggactaatcttagtcctcccccaagatgacatactctaacgttaccattgtcattatcccaataatctcctttagcaatagatctattatttacaacgaagtcagtaacattctcagtatatagctttttgttctcttgtttgaaatacaatcttccatcttcagctccaccataccagtcatttattcttaggtattttctagcccataggttttcagctgatagagccttatcaacctctagagatccgtctctagtagttatcctcatatcaaaatctttcttactaccctttaagtggaaatctaatataggacctagttccataactccatcatgtgatataaaagggatacctgcatagtcattactagctccagctaagtcccattcttttagtttattactgttagcagctgtagcggttttacctaaataagcactatcatggttatggtctgaggctgcagctcctatatcggatggcttaggtttattgaggttactataagctatacaccattcggaccatatgcctttaaaactacaaaacctagtatatgttttgccataactatctgtaaatagttgagttacctcaccccccttgggtaataccaatagagttccataaataccatatgtgtaaactacaggggagtttggtaaggtatctacactagatactgagtatatcccctcttccttacaaagattaaaatctactatatcatcttttctaatagttaaataaactccctcatgggtatggttagttggggatgcccccacatctgctgcagttggtttattatcttcatgatagaccttcttattgttcttattaacaatatccagagagtctatctttacaggccttccagcataccctatatggactttattatctgcatctatatagatcacatagtcatcactgccttctttagtcctacagctaaatccataattgtgggccccaataaatttctgacccggtctcatgattagatggcctgataattctccacccgtagtaggtaaggcaccaatatctgctggagtaggcttattttgtttactatatatttcagcccaattcgtccatccggtaccctcaatgtttgtagctgttctagtaaaaactcttccaccatctgcaaagaacatttgagaagcccagtgtcctgtattccaggataaaacaatcaatctcccatctgctaggattggggcatttctatcgacagaatttctaactgtagaataaatacctccctctgtaatggtgtttagatctacaccctctagtcttttggctgttttatcccaggccccaatatctgcgggtgttggcttagctccggagttataatcttttctccaagggaaccaatccgtattatttactttatacctccaatacttattaccattagtatcataatactcttgccatatccagttattagtattattatgcttagtctctgtactaacatatactatcagtataccatattttgtaccagttagtggggcattaggtaactcacctgagatcaggtattgcccctcagttaaagctgtattaaaatcagttatggcgtccttaggaatgggataagcctttaggtcagcaggggtaggcttattagcctcatcataaaccttataccacttactccaagaattatttcctgatgtgtagtttctaacatatctagttattttattggttgggtataggttaataaactcctgttggaatcccctctcacctgtatttctaaccataaaaaccctattactcatatgggctaaggttccctcgggggtatttttaaagtcaccagttcctgtatcaaagtagaagaaggcattcgcttgtttaaaggaattacaatctctatctaagggagcactaaccttaataagtgcttgatcttgattagcctttcggtctacttgattttgtaaactggtgtctttctcaaataataggtctaatctttttagcacatcctcaggggctagattataatcaggtactacattacccctagctaatatgaggtttagtacctttaatgaggtacttgaggttgcactctgtaccacaaattgtattttggtatcagtagctccagatggaatactaaatttatgagtttttaacttgtacccattactctgtggtgtactaccttgttttacaatactcctatattgttgacctccattagtgtaagccagtttaatttcatagctagtaaaactaccttcaatatcttctagaaaggctagtatataatcactatttggttctataggcagagttttaatctcaagagtttgtggacctgttgacataccagaccatttaaaacctcgtctctgggttggagtatctgtaatgggtgtgatattaccaggaccagtataagactcagagttgtaccactcaagcctattaatagtaccaacccttaaagcatctagcctatcctcattagacttagacttcttttctacctcagtcattttctgtttatgttcggtagcaaagttctcaatgttctcattgtccttgttaaaatcattcatttttggcttatctgttaactcccacttatttaaacctagggtaggagttttactagtacttggcattttgcatacctcctttattcagttatagcatattcttcccatttttcccaggtaagatctagactgtcccacttgctccacatataatcatatctatcgaacatctcccaagtaatataaagtaatataatttgatatattaggtgagcaggcattcttcccctgaatactctttctagagcctttaggttaggtggtacccctggtaggtcagtaaagctaatcttgatcttactctcttcagctatgaactctacctttacctttccacctgtataggccttagtaagatttttgatagatgtactattaaactttttccaagcagatagaactactgtaataatagctcttttctcttggtcagttggtgggtaatcaaagtatttatataactcaagatcagtaaaaaatctttctagaccttccttaggagtggtcttgggatccacatagtcttgtaattcctgtcccttagtatataacttctgaagttcagtagccataatggtgtttactaagttatcagcctcttttatattatcataaaattcaggaacatacaatagtaattctttttgaacctgttctagactatacataagttaccaccacctcagtaatggttggtatttgattagcaggaatagttaaagattgactacttccattaagtgtaatggttgtataatcttctactccctcaatatttaaaagcatagcccctattctatttatagataggctagtaattttaaatacttgactatttagaaattcttctagttctttcttgaagtttaattttatttgttcttctgtaactgaactcaatttcttaacttgagctcttacagtgatattaaaggtttgggctgactcaacagtaaaaacacatcctataggagctttaccctcacctaaacctttcttgcctggatccatgtattcttgaactttattaactagctcaggattagcaggcttattttcaactgtggttataatacctttagcagtatttattccatcccaacagggaagaaccacagctttacccactccagctacacttttacaccaatcagttaactgttgaacattcccatctccagatggttgtatagtggctttagtagctctttctcttaactcatcatctgtctcctgatctctaccaataacaagtatatctcccatagtagcacttctaagttctgctatagcattgataggaattaaatgtgtacctgttgatactttattgggtcctgaacctaaggtctcacattcaataatattaggctctatcacttgccagaaataatctcctccttggaatcttgaaccaacatcgggttcatagccaacaaatatagctgaccttctacacttagttggaattattctggatatccctacattggcagctctctcatctaagaacttacctgtagcagtacttagaaatactgagtctaatatttgattaacattaacagcataaaactcagctagcttaacagcaaaaaccatagccatatcataggtgaagcttccagttctagtgtcaatatcatcaggggataggcctatcatttcttctaataattctttatgtgttcgggagaataaatcttcagaaaatcccattatatcaccccttccagttttgtatctccatatatggtatttatccatacttcaatatatacattcttaccttgcacattatactttagatcagttactttagtcactctatcatcttctaagagacattcagggatagccctattaatctccatttcaagaagttcaggagttactagagagtcattaatcaaagctctaatatcacaaccataagaagtatcttgataaatcatataggcatttttaggagttattaatcttttatataaagattgttttaaggcctcaagaccatccacattatcataaatcctattaaggtttagatccagtttataggtcttggtattctccattgttttctcatcaactataagagtatctttaaagccattaggtagcattatatcaacctcctaagatccctaacataaaatatctttgtccatcatcatagggcataagataaacagtatcgccctcactaatagactcaatatgttttggaacatctataatatttccagatagtactaattttctattgtgaagacactcacattttagagggctagtactaagtaccttagctctataaatatttagaggggtggacatattactatatacttgttttacacagtctaataaattattagccattaaatatcaccctcctcagtacatttaagttttaaattcatggtgtagtcagtatcaaatttatgggtatcagactcaatgtagaaagccttgttaatttttaaatgtggtatactaaccacaatggctttgccactaatacaatcaggtacacctataacagttatagagatatcagttttaggtctcttacctgtttctagctttattctagccttctcatttaattgggcttggtttagttcatcactgatagtatcgtataattgaaatacaccatatttcttttggctgctatcatctttagcagaggcaaataaagtaatctcgggatcatctttacccttaccctgtttatatttacatactagctttacctggttgacaatactatcaaagtttctacttcttgaaaaggttccaatatttttaccatattcgaatttccacaattcattattggttcttcggtttataaaatcaaacttacctgtaatagaattatagtaaatataaaactgttctccagtttgttcataaacctcttttattaccttcttcataatatcatagggagtttgtttctcacatactaaactagagaaagtatatccagttttagctactactccaggggcaaccccaaaggctttacataatgactcaaatatagcttcgccagtttggttttcgaatacaaagctatctttattattagcccaataaatcatagggtcataagctttaaccttaagtaaatgctttttctcattatctgagatattcataataataccattaaagatattcttaccctcatggactagtactacctgatctccatcataaattggatgtatatcttgagcattatattggaatgatagggtacgaggggcagatgaagaagaccctgcccaactcttaccactggaggtatttgtaatatcaaaggatttatctccttgtaccacaattaattgcatattataacctccttatataatcaccagaactccaaccttctttatatcctgaaccattatctaatttatactttacataatgccatccattttgagatcttaatactgtaaagtgttcattaggccatatcttacccttagtgggattattgatacctggtccagttcttacccatagccatgagtaaacattagtagtagtagctgcccaaggttgagtacctccagaagaactacctcctgtattaccactataggctagtttaggttttggaattgtaaaactaactgatttaacctcaggcttcttatactcagttagttttatttttacttgaagagtaccaatatctccacctttctcagtatatgagatattatcaatagtaactaataagttaatatcagtactagtaatagtaaatcttactggatctttacccatttcaataagtttagcataacttactctagggtctgcaatatcagtatactcacatccatcgtagtatgagcttggtaactcaaaattaaaagaaaaagattttagcttagggtctcctatgaaagagagttcccctaagccttcaatggaaactgtactattatctctactatcagagatatttatatcagtgggatttactggtaacctaaacctagtatctccctgtattaaccagaattgatatttactatgcaaggtccagttcacctccctcgaacatttcctgatttaacatttccacaataaatctgtatactctcattaattcactttctgagattgttccatcttcagcctgtactgtgaaattaaatgagttgttaatgttcataactttagatccatcatcacttcctgctccagattgtcttagtaaatcctgagttttatctgcaggtaatacttgagagcctctaggcatttttgagaatgtaggacccataactaattcaggaccagcttcaccaaccatggcagctttatctgtaaagaagtcagtaccttcagcaagcattggtatctggggaatattaatacccttacccccaataataggtacccagtcaggtatcttaatagtattaagagcaccaattaagttattaatcataccaataatactattaataggagcttttgctagggataacataccttggaaaatacccccaaagatgttcttaacaccttcccaagctttagaccaattacctgtgaatactccagccacaaaagctattaaaccactcaacatctgcattaatccctgtagtattcctgatatagtttgaacggccccagtaacaactgaggagataacaggccatactgtttggaaagatgcggctaaaaggttaagtagtggagttagcatatccaccaacccttggaatatcataccaaaactctcaatagctgattgaatatatggaactacattctcagcaaagcttaagaacataggtagtagtgtattattccaccaatctgctagtccttgtaatattggcattaggaagttacctatagcttccacaacttgtgatatagctggggctatgtaggtgttaaaggcttcagctaatgatacagctattggcatgaaaacattagttatcaattctccaagagctgtaaaagtagcagagaacatagaacctaatacttctaatatagggcctaacacttccaatacagtttgccatacttgagtaaagccttgaacataaagaactactaagtctatggctggaattaggttattcataaatatagaagctaaagttccaaacatatcaagaagtacttgacctataggagctaatactcccatgataggctcagctaaaccattaaaggcttcttgtatattattattagcctctgataaataatctggtagacctattaagatctctccaaaattattatagatgtcttctccaagactccatatcttctcattaatttgatctgccacatcagcaggtaagaacttatataatatatcattggttagatctataaagggttgcatagcatccccaaactcccaaccattcatgatgtaatatatagtctctcctaaaccttggaaagcagaaacaaccattgagaatataggtcctagtttttcaaagccttcttgtataaatgtgataccatttagaacagcattagctataacctcaacggcaggggctagggcatctcccacatctaacataactacagcagctttggtttttattctctccatggttctattaaagcccttatccattttttcataggcagcttcagtggccccagcactatccttcatctcattaagagcattagtaaaggcctcagtaccttcaccagtcaaggctagtgcagctgaaccagcttctacagaaccaaagaggtcattgatacccagattacttttctgggcatgtttttctaacatctgaagggcctcttggatattacctccacctttaatgaagtctttgaagcccttaccagctatttcccggaagactttatcagtcttggttcccgatttagatagctcatctatagcagctcttatcttagtagtagctacagatgttggaaccccctgagctgttaatgcagctatagaggcagatacttcttcaaaagataccccagcagctgaggctgaaggtagcacattgaatagggattgtgatagttgctcaaagttagtcttaccaagtcttactgtagtaaacataaggtctgaggccctttgaacatccatattcttagctccatatgagttaataacagtagttagtccatcaaccgcagtttctattgatgtgataccacctatagaagctttaccagctgtttctaagaaactaaaaacgttatcctctggaactgatgaggatatagcttgataaagagcaggtactactttatcaggcaatatccctatatcagaacttaacttttttacctggccggacatcttatcaaaggtctcttgagtagagttgggtaatagagtcataacctcatttaaaccttgctcaaaatccccaaaggctttaacactgtccttagtaaaatcccagacagccttagctgagaatactccagcagctactccaccaattttggcaagagtacccatgaaggaattaccactatcagccatctggttaaatgcaccagagatcttatcttgggcagagaatatggcagtaaatgccgcttgacttgccattatatccctcctttatgattaagagcctttctttaacttatccctagcttttttatcttcctctaaagccagttcacatgaggctataagaaaggctttcctattgggagatagtttatcaaattcccagggtagtatattatgcttctggaataacacatgagcccaaaatgcactagtgtcggcctttattagttttttgcttctttgattagatcatccttattatcgcctaatccatttatgtccataacctcactagttattctagtgaaatctcctggtaagcttagtacatccataagtaaatctactggatccacaaacttagtagactctaaccattttggatctttaaagtcagggaatactattgtttctagtatcatttccctagtagctcttctttggtctgttattgagttagttatacctttgtttctagtaattactgtatttctcttttggatatcttccatttgcttagtagtgattggctttaatatccaaggtataggttggcccgctaattcatgaccctcagggaaactaaatctagctaccccttcaacttcaatttcgggtgattgtttacccttatcattttccatgaaaaattccatactaaattttgacataataatctacctccacaatattcttaatcttttataaatatcttacttctgaagctgagaatgatatttcttcttgaatttcttctccctcagcatctagtccaattagtggtaaatctccttctaattgtactcctagtaattgtactctgtcctcaccataattcttaacatagtcagaatctggatcatcacatacagcttgtatatccatcttagggaatataccagtttttaagtattccttaatagcttctcttatcattggagtagctttgaattgagttatagttccagttatatcataacctataacttttgaggttaatcctttctgacccataactcttttcttagtcacctcaggagtaaatagagcttctagttttattaagctagttacttgcttacctgatacaaaagctctaccctctctagcagacattctattaacttcactcatgggctatacctccttaattattcttaacagttacaaagtatttcttgaaagttcttacaggttgtgtaagtatagtagcatacatagtctttcctttactagcttcttcatctaccactacatcagagtcagggtccacattctttaatgctccttgagcttgtagtgtagttaatagacttattagtctatcctgagctagctttataccatctttgtggttagggaaaacattaggaactaagatctgagatcctagatctataacagcatccaatacagccacaactttgttatctgtaaagctttcatcccattcttctgtaaaagtatggtgtgtatttatatcttcctcaactactacctttactctttcagaatttgagtcagtttgagttgagaatataaattgacctgtttttaatccatcaactatttgagagtgttttagtcttggattggcatctactgctccaggatatgctttataagtaaggtcttcagtatatccagctgcagctctagcaccagctacccatgcagttgcttgagaagctgttaacttagtgcccccttctaatacaacaccattcttaacattgataatgtatgggtaatcacaagtagcaaagtcagaagtaactgccacaatattcttaccaacttcatctctgaagtatttaagttttgataatagagcagtgtgtaattcactatcagtaaatgggaaggccatagttttaaagttgtataactcacagttatctaagaagttgataacatcagagttattcatctgagtagaagtaccagtactaaactcagtcttagcagtctcatctatagaaccacttccacttactgtaaaccattgagacttaactgttgatatttcagttactcctgtagcctcaaagattttagatccctcaagatataataatatatcctttcctccaagaggattggtcttaatagttagagataacttattacccctttctccagctttagtagctgtaaatgttagagaccctactacagctttggctttagttccacctgttaggttatatactaaaacagttgcagcttcttttaaagcctctttaactagtaatacagtagggtgagttatgtcatacccaagttgatataatgcttctaggccaccttcattggttaccttgataacatctccagcattaccccatttaagttgtaatggtaagatcataactcctagattattaagcttaggctcattaagtccaccacttacgaatctagtatacataccaggtcttactttattttgtcctggaataaaagttcctcctgccatctattttacctccttctttagccagtcttttataatctgactagtttgttttattgttaactcttcatcaggtggaagggattgaactgcagcgttgaagacaaactcctcaacctggaaaagttgttgacaatgggctcttaattgaggtatggaaaatttttgtactttcactattttaccccctttgttatctcaaagttttcgaagtaagttggatctttataaagactaaccacaatatcatagtttatctctacctgagaatcttcttcagtttcaccttcaaatacttccacattctttattttgagatttttgttggtcttactaccatccctattaagtataggaatttttctatttctcaagtatatagcattagctatattctgagcaatttcaagagagtctttaggttcaaataccttaactcttaaagtattctcagttctataactacaaagagtatcattctgaggattaaataccttcttgaaatataatgagggatacttgaacttttcaggtattcgctcaaaatagaggatagtaattccagttagatcagatatgaatttagcaatactccctatatctgctgtcattaataactaccccctaaaacttcggctaaccaatcttctaattttctttggaaagcctgttcaaatattttttcatatatttttactgcattgtcccaataaggtttaccaggtactttcttttgtcttagtaccataccagtcttagctcctggttgataaataaatttatctcctgaccatatgccaggaacgaatctaaatgattgtccttgtggattagtgtagtgaccatcgtttacccacttagcatattttaggttagtaccaacttctaaagttagtcctccatcactacttacccatataccattcttacctcccttttgaaaggagttaagtaataatctagtgtctactacttgtagtctaattatttcatcttgaaccacatcaaggaagtctatccctgcagcttcaaaccatactgctaattgctttttgaaatcactattagctgcatctcttagcttctttataaacctttctatttgtttagcatctatttctatgcctccagaatttgaagccataactatctaaaatccttagcctctataccaaccttaatttttagacctcttatatccctaggagctttagctatatatgtgataccagtctcaaggtccacaattttatcattttgtctaacatcagttccaatagcaaaatctactgagtactcctgggtaatcttaaacctaggttctttgtactcaagtttttctagagttcctgacttaaaatgacagggtacctcagtcatgtctggctcatcaggataactaaagctaggggtatgggctagcccatatccgggatcttcagggtcttctaataggtggtatatattacatctatgatttaagagcttgttatatgaatttccaatcatattacagtacccttaatctcatagtagttgttctgatagatggactatcatcttctaagaaaggtttaatcagaggcataatatcaggctctatgacagccttatcagttcttcttgtatatgagtaatcatcataggtctcggattgaatatcagccttgctaatgaccaaggattgtagtccataatactcagcatacaatatatgggctaaccttaattctttactattaggatttttctccacaatagtatcatagtctttatttgaatttttaaaaattcctgagatcttggctttagctcttagtatatccatctcaatatttttggggtctcttttcttaatctcaggattacttgaaaagtcaattatttcatccggagtaatattcatatgagccacccctatctgtttcttttattcttgtttgtaaatcttctagcaggttcttctttactgtcatctgtagaaggtatttcttctccagtaaaatcttctagaggttcatcctcaacaggttcatctatgacaatcacatcatagttctgttttaaataatttactaggttatctttaacttcttctacatggtcttgagtaattctatgacccttaataaccagagtttgtaatttaccctttgctaatttgaccttagccataatatctctcctttctaatgaaaaagagcccacatttatagtgggccttcatgattaagcttttaccttgattatcttagcagcagctttaggatcttcaaacttaacatccatcttaagagttaaaactacataagtagctctttctctaggagctctttctaattcaattctgatatctcttgatatacctataactatattcttagggtgagttaagattatatctgatacttgagtagaagtatcttcataatcttgtagcatagctatacctttaacaggtacaccataagcagatttaacagagccatttataaatgagtcatcaccattagcagttaatctctctcctactaagtctacccaatcagtttctaaaccatttgagcagtagaatctccactcactggggtttcttaaatacttagctggtacagctttcttagcttgttttaataggtctttacttaaagcacccctttgagcatctactacatgagcagttaactgttttctaaccccatctaattgttgtaagaactcatcactaccctcactagtatcaccattaacaattatttcttccatatcaagagcaactctttcagctaataattgcattacagtgtcttctattgattttccttctatatttgtttctatagtatcatcagttaacttaaccacagctataaattctttagcttgtaaagtaactgttccagtagttggagctgaatatttagactcccctggatcttttccttcagttgcaggatttaatactctttgaccaaatcctattgactcaatctttttagagtctcctttcattggtacagttctagcctcttttaatattgttggctcatcaattatcattttaataaaagcgttagcttgttctgtgtttaatttacctccaccacttaatactgtagagttaaatactgctttatttattttagccataatcttttcctcctatcaattattcttggtttccaccaaataatccattaaatactgatttttgaacttcttgtccttctcctccatttttaacaatttgtttacttcctacatatggagccatggccttagctactgcctcagctattttttcttcctcagttttttcttcttgtttctggattaagccagcctctaacatagctttttccacagccttagcaactatatcttcagtagtagcttgttgaccttcactctttttaacttcaccctcaacaggtttagttccatctaatgcctttttgatagcttcgtctatcattttttgtacttgagtttcattcatctcttcttccccctccactgagtctaataattcattaatagcactttgtgctgtttttaacttttccacattttttgaagatattttcttacctgccttattgactggtaactcaaaggatttagctacttcctcgggagttcctaataatattccctccatagtttcagaaaattcttgaagagcttcctttatcttatctacatcactttcaaaagatctagtgtaatcccaactagaatatggatatagaatatcttctaaggtactaactgcattccagaaattatccctttttgcagtctctttatatttttcagagtatgcacctttctgtatatgctttggagttaaccctaaggcctttccaatcttatcaagtatagattgacctatagacttctcaatctcatcaatatctacatcttgtgtagaatatttaccagtaccacccatagaccatccagtaatttcgcctttctcaatcttgctccatagatcatcatcgacaatctcagctttagctagccaagttccagctttaactactgtaccttctattgtagtatcttcctcagttacccatgattttacaatcttgacaccctcaagagtgttctcattgtgttgtaaatcactaccaaggccattttcattaaaccactcacaagctttcttgatctcttcctcagtcataaaattatcatggtagtcagcagtcattggctcatatactacaccgataacaaaatgattatctccttcagactcagactttaagattggcttatcatatctaaatctattaggagccccaagttctttagccacaatccattgccatttattagctgctttatcaactaatgaaaggtaatcaattttagcatctgagatctcaatagctttcttaactgattttactggcatttactctccctcctttacaaattatattctgctatcacttgatctctgatagcttctttttcttctttagataatcctagtatatccttatcaattacaggcccatgggtacaatgacaattcacagtctcagaagctggtaagttgatatccctaggaaatctagcttcataaattcctacagtgaagtactcacctttattaatgacagtaccatccagatcgacatggtgttgccttgggtgaataccccttccccctgagtgtttccactgtattcctgttactgcggggcattgattaaaagcctcatccttagcatatgaatgagctcttaacatttcagtaatagcagtagctctagctctagttctactaaagccataagtctcagataatttaccaactacatcttctacagactctccatcttcaagagccttatccagaatattctgtagtttttcatgggaagttaatttcatcatttcccctagtttagaagaccactcatctataaaggtagtagtatatggagaaaagactttggttagggataagtccttatcaataccttgtaaataagtatctcctaaattttctatagcttcttgataacaactcttaagagtttctgctaaagaagtatcgatattatctgtacctatttgagactccacatattccataaattcttcaatggtttcaaagtctccatcttttataagatgttttaattcttctgtaaggagatcagaaatagtgtcttctaattcagagatcttttctattgtataatcaatctcctcatagccagcttctttcaattctttcttaaggctatcatcttcattctttaagatcttatcaattttagcgatcaactcatcagtacccactattacttacctccttttaattgatagtttaataactgtttcttagcctctttaagtacagctatcacctcatcactcccattagagctttgagccttctcaattatacttgttaagttattactcattgaagaggcaactgagtaagtagggatatttgcccattcttcatcaataggagtatagtccttattgattgatgaatagtactcctcattaatctgattaggagtcatagctctagaggctatagcaaacattcctttctgataatcagagttctcaatattaggactcttaaagtaagcttccacatatttaaaaccatagccagatagaataacattatttagtatccatgttaggttttctctttcaggaacaaatacttgctcttcagtttttcttgtagcctctctggctgtagccacattataatcttgggagtaccctacatatatatctggtagtaagaaagaagattgtatctttttcctagtattatccatgtagtcttggaataactcatccttctgtaatatttcagataggggcttgacctcaacagtaactggcttagaatcatcaagggcagtgtctctctctgcagcttcagtttctaatactaagaaaccatgctgggaattttcaccttttacattattcatgtactcagttaattcattccaagatttatcattaagagtaccaccttgaattagtaacattaatggagtatgtttaccattagtaaaatatctccagtttaataattcggcctttcttgaaccttgagcggctaacataggaccttcccatcttggtgtaccatagacaccataacctgttttaaaatgaagtatactgttagctcgatctttaagaggtatctctcccttttcataatactttccagtattcatatctagatctctaggatctccccactctttaaagaagattgattgattatttacagtctgcttaaatcttctgaacctttttcttctagtgtactgtttaccatatcgggttacagtgtactctgtactctcatcatctagcttaagaattttaattgtcttagggtcttcaatttcttttatctcttttacgagagct